European Patent Specification EP 3 836 908 B1, published June 11, 2025. Title: NUCLEIC ACIDS AND NUCLEIC ACID ANALOGS FOR TREATING, PREVENTING, AND DISRUPTING PATHOLOGICAL POLYNUCLEOTIDE-BINDING PROTEIN INCLUSIONS. Applicant: UNIVERSITY OF PITTSBURGH-OF THE COMMONWEALTH SYSTEM OF HIGHER EDUCATION. The sequence listing filed with the application follows.

SEQUENCE LISTING (121 sequences)

SEQ ID NO: 1 - protein, 414 aa, Homo sapiens
MSEYIRVTEDENDEPIEIPSEDDGTVLLSTVTAQFPGACGLRYRNPVSQCMRGVRLVEGILHAPDAGWGNLVYVVNYPKDNKRKMDETDASSAVKVKRAVQKTSDLIVLGLPWKTTEQDLKEYFSTFGEVLMVQVKKDLKTGHSKGFGFVRFTEYETQVKVMSQRHMIDGRWCDCKLPNSKQSQDEPLRSRKVFVGRCTEDMTEDELREFFSQYGDVMDVFIPKPFRAFAFVTFADDQIAQSLCGEDLIIKGISVHISNAEPKHNSNRQLERSGRFGGNPGGFGNQGGFGNSRGGGAGLGNNQGSNMGGGMNFGAFSINPAMMAAAQAALQSSWGMMGMLASQQNQSGPSGNNQNQGNMQREPNQAFGSGNNSYSGSNSGAAIGWGSASNAGSGSGFNGGFGSSMDSKSSGWGM

SEQ ID NO: 2 - protein, 526 aa, Homo sapiens
MASNDYTQQATQSYGAYPTQPGQGYSQQSSQPYGQQSYSGYSQSTDTSGYGQSSYSSYGQSQNTGYGTQSTPQGYGSTGGYGSSQSSQSSYGQQSSYPGYGQQPAPSSTSGSYGSSSQSSSYGQPQSGSYSQQPSYGGQQQSYGQQQSYNPPQGYGQQNQYNSSSGGGGGGGGGGNYGQDQSSMSSGGGSGGGYGNQDQSGGGGSGGYGQQDRGGRGRGGSGGGGGGGGGGYNRSSGGYEPRGRGGGRGGRGGMGGSDRGGFNKFGGPRDQGSRHDSEQDNSDNNTIFVQGLGENVTIESVADYFKQIGIIKTNKKTGQPMINLYTDRETGKLKGEATVSFDDPPSAKAAIDWFDGKEFSGNPIKVSFATRRADFNRGGGNGRGGRGRGGPMGRGGYGGGGSGGGGRGGFPSGGGGGGGQQRAGDWKCPNPTCENMNFSWRNECNQCKAPKPDGPGGGPGGSHMGGNYGDDRRGGRGGYDRGGYRGRGGDRGGFRGGRGGGDRGGFGPGKMDSRGEHRQDRRERPY

SEQ ID NO: 3 - protein, 758 aa, Homo sapiens
MAEPRQEFEVMEDHAGTYGLGDRKDQGGYTMHQDQEGDTDAGLKESPLQTPTEDGSEEPGSETSDAKSTPTAEDVTAPLVDEGAPGKQAAAQPHTEIPEGTTAEEAGIGDTPSLEDEAAGHVTQEPESGKVVQEGFLREPGPPGLSHQLMSGMPGAPLLPEGPREATRQPSGTGPEDTEGGRHAPELLKHQLLGDLHQEGPPLKGAGGKERPGSKEEVDEDRDVDESSPQDSPPSKASPAQDGRPPQTAAREATSIPGFPAEGAIPLPVDFLSKVSTEIPASEPDGPSVGRAKGQDAPLEFTFHVEITPNVQKEQAHSEEHLGRAAFPGAPGEGPEARGPSLGEDTKEADLPEPSEKQPAAAPRGKPVSRVPQLKARMVSKSKDGTGSDDKKAKTSTRSSAKTLKNRPCLSPKHPTPGSSDPLIQPSSPAVCPEPPSSPKYVSSVTSRTGSSGAKEMKLKGADGKTKIATPRGAAPPGQKGQANATRIPAKTPPAPKTPPSSGEPPKSGDRSGYSSPGSPGTPGSRSRTPSLPTPPTREPKKVAVVRTPPKSPSSAKSRLQTAPVPMPDLKNVKSKIGSTENLKHQPGGGKVQIINKKLDLSNVQSKCGSKDNIKHVPGGGSVQIVYKPVDLSKVTSKCGSLGNIHHKPGGGQVEVKSEKLDFKDRVQSKIGSLDNITHVPGGGNKKIETHKLTFRENAKAKTDHGAEIVYKSPVVSGDTSPRHLSNVSSTGSIDMVDSPQLATLADEVSASLAKQGL

SEQ ID NO: 4 - DNA, 3789 bp, Artificial Sequence
  Synthetic construct
atgaagatggacaaaaagactatagtttggtttagaagagacctaaggattgaggataatcctgcattagcagcagctgctcacgaaggatctgtttttcctgtcttcatttggtgtcctgaagaagaaggacagttttatcctggaagagcttcaagatggtggatgaaacaatcacttgctcacttatctcaatccttgaaggctcttggatctgacctcactttaatcaaaacccacaacacgatttcagcgatcttggattgtatccgcgttaccggtgctacaaaagtcgtctttaaccacctctatgatcctgtttcgttagttcgggaccataccgtaaaggagaagctggtggaacgtgggatctctgtgcaaagctacaatggagatctattgtatgaaccgtgggagatatactgcgaaaagggcaaaccttttacgagtttcaattcttactggaagaaatgcttagatatgtcgattgaatccgttatgcttcctcctccttggcggttgatgccaataactgcagcggctgaagcgatttgggcgtgttcgattgaagaactagggctggagaatgaggccgagaaaccgagcaatgcgttgttaactagagcttggtctccaggatggagcaatgctgataagttactaaatgagttcatcgagaagcagttgatagattatgcaaagaacagcaagaaagttgttgggaattctacttcactactttctccgtatctccatttcggggaaataagcgtcagacacgttttccagtgtgcccggatgaaacaaattatatgggcaagagataagaacagtgaaggagaagaaagtgcagatctttttcttaggggaatcggtttaagagagtattctcggtatatatgtttcaacttcccgtttactcacgagcaatcgttgttgagtcatcttcggtttttcccttgggatgctgatgttgataagttcaaggcctggagacaaggcaggaccggttatccgttggtggatgccggaatgagagagctttgggctaccggatggatgcataacagaataagagtgattgtttcaagctttgctgtgaagtttcttctccttccatggaaatggggaatgaagtatttctgggatacacttttggatgctgatttggaatgtgacatccttggctggcagtatatctctgggagtatccccgatggccacgagcttgatcgcttggacaatcccgcgttacaaggcgccaaatatgacccagaaggtgagtacataaggcaatggcttcccgagcttgcgagattgccaactgaatggatccatcatccatgggacgctcctttaaccgtactcaaagcttctggtgtggaactcggaacaaactatgcgaaacccattgtagacatcgacacagctcgtgagctactagctaaagctatttcaagaacccgtggagcacagatcatgatcggagcagcagccctcatggtgagcaagggcgaggaggataacatggccatcatcaaggagttcatgcgcttcaaggtgcacatggagggctccgtgaacggccacgagttcgagatcgagggcgagggcgagggccgcccctacgagggcacccagaccgccaagctgaaggtgaccaagggtggccccctgcccttcgcctgggacatcctgtcccctcagttcatgtacggctccaaggcctacgtgaagcaccccgccgacatccccgactacttgaagctgtccttccccgagggcttcaagtgggagcgcgtgatgaacttcgaggacggcggcgtggtgaccgtgacccaggactcctccctgcaggacggcgagttcatctacaaggtgaagctgcgcggcaccaacttcccctccgacggccccgtaatgcagaagaagaccatgggctgggaggcctcctccgagcggatgtaccccgaggacggcgccctgaagggcgagatcaagcagaggctgaagctgaaggacggcggccactacgacgctgaggtcaagaccacctacaaggccaagaagcccgtgcagctgcccggcgcctacaacgtcaacatcaagttggacatcacctcccacaacgaggactacaccatcgtggaacagtacgaacgcgccgagggccgccactccaccggcggcatggacgagctgtacaagatggcctcaaacgattatacccaacaagcaacccaaagctatggggcctaccccacccagcccgggcagggctattcccagcagagcagtcagccctacggacagcagagttacagtggttatagccagtccacggacacttcaggctatggccagagcagctattcttcttatggccagagccagaacacaggctatggaactcagtcaactccccagggatatggctcgactggcggctatggtagtagccagagctcccaatcgtcttacgggcagcagtcctcctatcctggctatggccagcagccagctcccagcagcacctcgggaagttacggtagcagttctcagagcagcagctatgggcagccccagagtgggagctacagccagcagcctagctatggtggacagcagcaaagctatggacagcagcaaagctataatccccctcagggctatggacagcagaaccagtacaacagcagcagtggtggtggaggtggaggtggaggtggaggtaactatggccaagatcaatcctccatgagtagtggtggtggcagtggtggcggttatggcaatcaagaccagagtggtggaggtggcagcggtggctatggacagcaggaccgtggaggccgcggcaggggtggcagtggtggcggcggcggcggcggcggtggtggttacaaccgcagcagtggtggctatgaacccagaggtcgtggaggtggccgtggaggcagaggtggcatgggcggaagtgaccgtggtggcttcaataaatttggtggccctcgggaccaaggatcacgtcatgactccgaacaggataattcagacaacaacaccatctttgtgcaaggcctgggtgagaatgttacaattgagtctgtggctgattacttcaagcagattggtattattaagacaaacaagaaaacgggacagcccatgattaatttgtacacagacagggaaactggcaagctgaagggagaggcaacggtctcttttgatgacccaccttcagctaaagcagctattgactggtttgatggtaaagaattctccggaaatcctatcaaggtctcatttgctactcgccgggcagactttaatcggggtggtggcaatggtcgtggaggccgagggcgaggaggacccatgggccgtggaggctatggaggtggtggcagtggtggtggtggccgaggaggatttcccagtggaggtggtggcggtggaggacagcagcgagctggtgactggaagtgtcctaatcccacctgtgagaatatgaacttctcttggaggaatgaatgcaaccagtgtaaggcccctaaaccagatggcccaggagggggaccaggtggctctcacatggggggtaactacggggatgatcgtcgtggtggcagaggaggctatgatcgaggcggctaccggggccgcggcggggaccgtggaggcttccgagggggccggggtggtggggacagaggtggctttggccctggcaagatggattccaggggtgagcacagacaggatcgcagggagaggccgtattaa

SEQ ID NO: 5 - protein, 1262 aa, Artificial Sequence
  Synthetic construct
MKMDKKTIVWFRRDLRIEDNPALAAAAHEGSVFPVFIWCPEEEGQFYPGRASRWWMKQSLAHLSQSLKALGSDLTLIKTHNTISAILDCIRVTGATKVVFNHLYDPVSLVRDHTVKEKLVERGISVQSYNGDLLYEPWEIYCEKGKPFTSFNSYWKKCLDMSIESVMLPPPWRLMPITAAAEAIWACSIEELGLENEAEKPSNALLTRAWSPGWSNADKLLNEFIEKQLIDYAKNSKKVVGNSTSLLSPYLHFGEISVRHVFQCARMKQIIWARDKNSEGEESADLFLRGIGLREYSRYICFNFPFTHEQSLLSHLRFFPWDADVDKFKAWRQGRTGYPLVDAGMRELWATGWMHNRIRVIVSSFAVKFLLLPWKWGMKYFWDTLLDADLECDILGWQYISGSIPDGHELDRLDNPALQGAKYDPEGEYIRQWLPELARLPTEWIHHPWDAPLTVLKASGVELGTNYAKPIVDIDTARELLAKAISRTRGAQIMIGAAALMVSKGEEDNMAIIKEFMRFKVHMEGSVNGHEFEIEGEGEGRPYEGTQTAKLKVTKGGPLPFAWDILSPQFMYGSKAYVKHPADIPDYLKLSFPEGFKWERVMNFEDGGVVTVTQDSSLQDGEFIYKVKLRGTNFPSDGPVMQKKTMGWEASSERMYPEDGALKGEIKQRLKLKDGGHYDAEVKTTYKAKKPVQLPGAYNVNIKLDITSHNEDYTIVEQYERAEGRHSTGGMDELYKMASNDYTQQATQSYGAYPTQPGQGYSQQSSQPYGQQSYSGYSQSTDTSGYGQSSYSSYGQSQNTGYGTQSTPQGYGSTGGYGSSQSSQSSYGQQSSYPGYGQQPAPSSTSGSYGSSSQSSSYGQPQSGSYSQQPSYGGQQQSYGQQQSYNPPQGYGQQNQYNSSSGGGGGGGGGGNYGQDQSSMSSGGGSGGGYGNQDQSGGGGSGGYGQQDRGGRGRGGSGGGGGGGGGGYNRSSGGYEPRGRGGGRGGRGGMGGSDRGGFNKFGGPRDQGSRHDSEQDNSDNNTIFVQGLGENVTIESVADYFKQIGIIKTNKKTGQPMINLYTDRETGKLKGEATVSFDDPPSAKAAIDWFDGKEFSGNPIKVSFATRRADFNRGGGNGRGGRGRGGPMGRGGYGGGGSGGGGRGGFPSGGGGGGGQQRAGDWKCPNPTCENMNFSWRNECNQCKAPKPDGPGGGPGGSHMGGNYGDDRRGGRGGYDRGGYRGRGGDRGGFRGGRGGGDRGGFGPGKMDSRGEHRQDRRERPY

SEQ ID NO: 6 - DNA, 1770 bp, Artificial Sequence
  Synthetic construct
atgggtaagcctatccctaaccctctcctcggtctcgattcaacaagtttgatgtctgaatatattcgggtaaccgaagatgagaacgatgagcccattgaaataccatcggaagacgatgggacggtgctgctctccacggttacagcccagtttccaggggcgtgtgggcttcgctacaggaatccagtgtctcagtgtatgagaggtgtccggctggtagaaggaattctgcatgccccagatgctggctggggaaatctggtgtatgttgtcaactatccaaaagataacaaaagaaaaatggatgagacagatgcttcatcagcagtgaaagtgaaaagagcagtccagaaaacatccgatttaatagtgttgggtctcccatggaaaacaaccgaacaggacctgaaagagtattttagtacctttggagaagttcttatggtgcaggtcaagaaagatcttaagactggtcattcaaaggggtttggctttgttcgttttacggaatatgaaacacaagtgaaagtaatgtcacagcgacatatgatagatggacgatggtgtgactgcaaacttcctaattctaagcaaagccaagatgagcctttgagaagcagaaaagtgtttgtggggcgctgtacagaggacatgactgaggatgagctgcgggagttcttctctcagtacggggatgtgatggatgtcttcatccccaagccattcagggcctttgcctttgttacatttgcagatgatcagattgcgcagtctctttgtggagaggacttgatcattaaaggaatcagcgttcatatatccaatgccgaacctaagcacaatagcaatagacagttagaaagaagtggaagatttggtggtaatccaggtggctttgggaatcagggtggatttggtaatagcagagggggtggagctggtttgggaaacaatcaaggtagtaatatgggtggtgggatgaactttggtgcgttcagcattaatccagccatgatggctgccgcccaggcagcactacagagcagttggggtatgatgggcatgttagccagccagcagaaccagtcaggcccatcgggtaataaccaaaaccaaggcaacatgcagagggagccaaaccaggccttcggttctggaaataactcttatagtggctctaattctggtgcagcaattggttggggatcagcatccaatgcagggtcgggcagtggttttaatggaggctttggctcaagcatggattctaagtcttctggctggggaatgggcagttcaggatcatccgggcacactctctacgccccaggcgggtacgatattatgggctggctgatccagatcatgaacaggcccaatccccaggtcgagctgggacccgtggatacttcatgtgcactggtgctgtgcgacctgaagcagaaggatacccccgtggtgtacgcatccgaagcgttcctctacatgaccgggtactcgaacgcggaggtgctgggtcgcaactgccggttcctgcagagccccgacggaatggtcaagcccaagtccactcggaaatacgtggattccaacaccatcaatactatgaggaaggctatcgataggaacgcggaagtccaagtggaggtggtgaacttcaagaagaatggccagagattcgtcaatttccttaccatgatccctgtgcgcgatgagactggagagtaccgatactcaatgggcttccagtgtgaaaccgagtgttaa

SEQ ID NO: 7 - protein, 589 aa, Artificial Sequence
  Synthetic construct
MGKPIPNPLLGLDSTSLMSEYIRVTEDENDEPIEIPSEDDGTVLLSTVTAQFPGACGLRYRNPVSQCMRGVRLVEGILHAPDAGWGNLVYVVNYPKDNKRKMDETDASSAVKVKRAVQKTSDLIVLGLPWKTTEQDLKEYFSTFGEVLMVQVKKDLKTGHSKGFGFVRFTEYETQVKVMSQRHMIDGRWCDCKLPNSKQSQDEPLRSRKVFVGRCTEDMTEDELREFFSQYGDVMDVFIPKPFRAFAFVTFADDQIAQSLCGEDLIIKGISVHISNAEPKHNSNRQLERSGRFGGNPGGFGNQGGFGNSRGGGAGLGNNQGSNMGGGMNFGAFSINPAMMAAAQAALQSSWGMMGMLASQQNQSGPSGNNQNQGNMQREPNQAFGSGNNSYSGSNSGAAIGWGSASNAGSGSGFNGGFGSSMDSKSSGWGMGSSGSSGHTLYAPGGYDIMGWLIQIMNRPNPQVELGPVDTSCALVLCDLKQKDTPVVYASEAFLYMTGYSNAEVLGRNCRFLQSPDGMVKPKSTRKYVDSNTINTMRKAIDRNAEVQVEVVNFKKNGQRFVNFLTMIPVRDETGEYRYSMGFQCETEC

SEQ ID NO: 8 - DNA, 1824 bp, Artificial Sequence
  Synthetic construct
atgcacactctctacgccccaggcgggtacgatattatgggctggctgatccagatcatgaacaggcccaatccccaggtcgagctgggacccgtggatacttcatgtgcactggtgctgtgtgaccttaagcagaaggacacccctgtggtgtacgcctccgaagcattcctgtacatgaccgggtactcgaacgccgaagtgctgggacggaactgccgcttcctgcaatccccggatggaatggtgaagcctaagtcaacccgcaaatacgtggactccaacactatcaacaccatgcgcaaggccattgaccgcaatgctgaggtgcaagtggaagtggtgaacttcaagaagaacggacagcgcttcgtcaacttcctgactatgattcccgtgcgggacgaaaccggcgaataccggtacagcatggggtttcagtgcgagactgagggctccggcggcagcggtggctccggaggcagcggaggtaccggcggcagtggagggtctggtggcagcggaatgtctgaatatattcgggtaaccgaagatgagaacgatgagcccattgaaataccatcggaagacgatgggacggtgctgctctccacggttacagcccagtttccaggggcgtgtgggcttcgctacaggaatccagtgtctcagtgtatgagaggtgtccggctggtagaaggaattctgcatgccccagatgctggctggggaaatctggtgtatgttgtcaactatccaaaagataacaaaagaaaaatggatgagacagatgcttcatcagcagtgaaagtgaaaagagcagtccagaaaacatccgatttaatagtgttgggtctcccatggaaaacaaccgaacaggacctgaaagagtattttagtacctttggagaagttcttatggtgcaggtcaagaaagatcttaagactggtcattcaaaggggtttggctttgttcgttttacggaatatgaaacacaagtgaaagtaatgtcacagcgacatatgatagatggacgatggtgtgactgcaaacttcctaattctaagcaaagccaagatgagcctttgagaagcagaaaagtgtttgtggggcgctgtacagaggacatgactgaggatgagctgcgggagttcttctctcagtacggggatgtgatggatgtcttcatccccaagccattcagggcctttgcctttgttacatttgcagatgatcagattgcgcagtctctttgtggagaggacttgatcattaaaggaatcagcgttcatatatccaatgccgaacctaagcacaatagcaatagacagttagaaagaagtggaagatttggtggtaatccaggtggctttgggaatcagggtggatttggtaatagcagagggggtggagctggtttgggaaacaatcaaggtagtaatatgggtggtgggatgaactttggtgcgttcagcattaatccagccatgatggctgccgcccaggcagcactacagagcagttggggtatgatgggcatgttagccagccagcagaaccagtcaggcccatcgggtaataaccaaaaccaaggcaacatgcagagggagccaaaccaggccttcggttctggaaataactcttatagtggctctaattctggtgcagcaattggttggggatcagcatccaatgcagggtcgggcagtggttttaatggaggctttggctcaagcatggattctaagtcttctggctggggaatgcttggtaccatgggtaagcctatccctaaccctctcctcggtctcgattcaacataa

SEQ ID NO: 9 - protein, 607 aa, Artificial Sequence
  Synthetic construct
MHTLYAPGGYDIMGWLIQIMNRPNPQVELGPVDTSCALVLCDLKQKDTPVVYASEAFLYMTGYSNAEVLGRNCRFLQSPDGMVKPKSTRKYVDSNTINTMRKAIDRNAEVQVEVVNFKKNGQRFVNFLTMIPVRDETGEYRYSMGFQCETEGSGGSGGSGGSGGTGGSGGSGGSGMSEYIRVTEDENDEPIEIPSEDDGTVLLSTVTAQFPGACGLRYRNPVSQCMRGVRLVEGILHAPDAGWGNLVYVVNYPKDNKRKMDETDASSAVKVKRAVQKTSDLIVLGLPWKTTEQDLKEYFSTFGEVLMVQVKKDLKTGHSKGFGFVRFTEYETQVKVMSQRHMIDGRWCDCKLPNSKQSQDEPLRSRKVFVGRCTEDMTEDELREFFSQYGDVMDVFIPKPFRAFAFVTFADDQIAQSLCGEDLIIKGISVHISNAEPKHNSNRQLERSGRFGGNPGGFGNQGGFGNSRGGGAGLGNNQGSNMGGGMNFGAFSINPAMMAAAQAALQSSWGMMGMLASQQNQSGPSGNNQNQGNMQREPNQAFGSGNNSYSGSNSGAAIGWGSASNAGSGSGFNGGFGSSMDSKSSGWGMLGTMGKPIPNPLLGLDST

SEQ ID NO: 10 - RNA, 24 nt, Artificial Sequence
  Synthetic construct
ugugugugugugugugugugugug

SEQ ID NO: 11 - DNA, 112 bp, Artificial Sequence
  Synthetic construct
cmgmcmgmcmgmcmgmcmgmcmgmcmgmcmgmtmgmtmgmtmgmtmgmtmgmtmgmtmgmtmgmtmgmtmgmtmgmtmgmcmgmcmgmcmgmcmgmcmgmcmgmcmgmcmgm

SEQ ID NO: 12 - RNA, 56 nt, Artificial Sequence
  Synthetic construct
cgcgcgcgcgcgcgcgugugugugugugugugugugugugcgcgcgcgcgcgcgcg

SEQ ID NO: 13 - RNA, 68 nt, Artificial Sequence
  Synthetic construct
gmamgmamgmamgmcmgmcmgmumgmcmamgmamgmamcmumumgmgmumgmgmumgmcmamumamam

SEQ ID NO: 14 - RNA, 34 nt, Artificial Sequence
  Synthetic construct
gagagagcgcgugugugugugugguggugcauaa

SEQ ID NO: 15 - DNA, 29 bp, Unknown
  natural sequence
gttcttttgttttgttttttaacacttgt

SEQ ID NO: 16 - DNA, 33 bp, Unknown
  natural sequence
ttaagtgagtttttgttcttagataacccacat

SEQ ID NO: 17 - DNA, 25 bp, Unknown
  natural sequence
ttgtggtgtgctttgcaggaggact

SEQ ID NO: 18 - DNA, 37 bp, Unknown
  natural sequence
ttaaataaaactgatttaaataatatgtgtctttgtt

SEQ ID NO: 19 - RNA, 29 nt, Unknown
  natural sequence
guucuuuuguuuuguuuuuuaacacuugu

SEQ ID NO: 20 - RNA, 33 nt, Unknown
  natural sequence
uuaagugaguuuuuguucuuagauaacccacau

SEQ ID NO: 21 - RNA, 25 nt, Unknown
  natural sequence
uuguggugugcuuugcaggaggacu

SEQ ID NO: 22 - RNA, 37 nt, Unknown
  natural sequence
uuaaauaaaacugauuuaaauaauaugugucuuuguu

SEQ ID NO: 23 - DNA, 286 bp, Unknown
  natural sequence
acccccatttccttaattatttcaggaataattctcccgaaatcaggtcaaccccatcaccaaccaaccaaccagttgagttccagattctatgtgaattaaaaagtcaatatatgtataattctgagatgacttaggttggacattcaatgttgtgctatgaatttcctctttatgcagagtatctgtttgcttgcagagtggctttctggcttgctgccagcctgtgcatggaccacgcttatgagttcaggatctacggcaatgtgaatcattcagatgttta

SEQ ID NO: 24 - DNA, 35 bp, Unknown
  natural sequence
ttggacattcaatgttgtgctatgaatttcctctt

SEQ ID NO: 25 - RNA, 286 nt, Unknown
  natural sequence
acccccauuuccuuaauuauuucaggaauaauucucccgaaaucaggucaaccccaucaccaaccaaccaaccaguugaguuccagauucuaugugaauuaaaaagucaauauauguauaauucugagaugacuuagguuggacauucaauguugugcuaugaauuuccucuuuaugcagaguaucuguuugcuugcagaguggcuuucuggcuugcugccagccugugcauggaccacgcuuaugaguucaggaucuacggcaaugugaaucauucagauguuua

SEQ ID NO: 26 - RNA, 35 nt, Unknown
  natural sequence
uuggacauucaauguugugcuaugaauuuccucuu

SEQ ID NO: 27 - DNA, 23 bp, Unknown
  natural sequence
gattaaaagttgtgttccccaat

SEQ ID NO: 28 - RNA, 23 nt, Unknown
  natural sequence
gauuaaaaguuguguuccccaau

SEQ ID NO: 29 - DNA, 46 bp, Unknown
  natural sequence
gagacctggttgtgtgtgtgtgagtggttgaccttcctccatcccc

SEQ ID NO: 30 - RNA, 46 nt, Unknown
  natural sequence
gagaccugguugugugugugugagugguugaccuuccuccaucccc

SEQ ID NO: 31 - DNA, 28 bp, Unknown
  natural sequence
gtgtttgtgtgtgtgcgcgtgtgcgttc

SEQ ID NO: 32 - RNA, 28 nt, Unknown
  natural sequence
guguuugugugugugcgcgugugcguuc

SEQ ID NO: 33 - DNA, 12 bp, Artificial Sequence
  Synthetic construct
  repeat_unit (1)..(12)
atgtgtgtgtgt

SEQ ID NO: 34 - DNA, 12 bp, Artificial Sequence
  Synthetic construct
  repeat_unit (1)..(12)
gtatgtgtgtgt

SEQ ID NO: 35 - DNA, 12 bp, Artificial Sequence
  Synthetic construct
  repeat_unit (1)..(12)
gtgtatgtgtgt

SEQ ID NO: 36 - DNA, 12 bp, Artificial Sequence
  Synthetic construct
  repeat_unit (1)..(12)
gtgtgtatgtgt

SEQ ID NO: 37 - DNA, 12 bp, Artificial Sequence
  Synthetic construct
  repeat_unit (1)..(12)
gtgtgtgtgtat

SEQ ID NO: 38 - DNA, 12 bp, Artificial Sequence
  Synthetic construct
  repeat_unit (1)..(12)
tatgtgtgtgtg

SEQ ID NO: 39 - DNA, 12 bp, Artificial Sequence
  Synthetic construct
  repeat_unit (1)..(12)
tgtatgtgtgtg

SEQ ID NO: 40 - DNA, 12 bp, Artificial Sequence
  Synthetic construct
  repeat_unit (1)..(12)
tgtgtatgtgtg

SEQ ID NO: 41 - DNA, 12 bp, Artificial Sequence
  Synthetic construct
  repeat_unit (1)..(12)
tgtgtatgtgtg

SEQ ID NO: 42 - DNA, 12 bp, Artificial Sequence
  Synthetic construct
  repeat_unit (1)..(12)
tgtgtgtatgtg

SEQ ID NO: 43 - DNA, 12 bp, Artificial Sequence
  Synthetic construct
  repeat_unit (1)..(12)
tgtgtgtgtatg

SEQ ID NO: 44 - DNA, 12 bp, Artificial Sequence
  Synthetic construct
  repeat_unit (1)..(12)
tgtgtgtgtgta

SEQ ID NO: 45 - RNA, 12 nt, Artificial Sequence
  Synthetic construct
  repeat_unit (1)..(12)
augugugugugu

SEQ ID NO: 46 - RNA, 12 nt, Artificial Sequence
  Synthetic construct
  repeat_unit (1)..(12)
guaugugugugu

SEQ ID NO: 47 - RNA, 12 nt, Artificial Sequence
  Synthetic construct
  repeat_unit (1)..(12)
guguaugugugu

SEQ ID NO: 48 - RNA, 12 nt, Artificial Sequence
  Synthetic construct
  repeat_unit (1)..(12)
guguguaugugu

SEQ ID NO: 49 - RNA, 12 nt, Artificial Sequence
  Synthetic construct
  repeat_unit (1)..(12)
guguguguguau

SEQ ID NO: 50 - RNA, 12 nt, Artificial Sequence
  Synthetic construct
  repeat_unit (1)..(12)
uaugugugugug

SEQ ID NO: 51 - RNA, 12 nt, Artificial Sequence
  Synthetic construct
  repeat_unit (1)..(12)
uguaugugugug

SEQ ID NO: 52 - RNA, 12 nt, Artificial Sequence
  Synthetic construct
  repeat_unit (1)..(12)
uguguaugugug

SEQ ID NO: 53 - RNA, 12 nt, Artificial Sequence
  Synthetic construct
  repeat_unit (1)..(12)
uguguaugugug

SEQ ID NO: 54 - RNA, 12 nt, Artificial Sequence
  Synthetic construct
  repeat_unit (1)..(12)
uguguguaugug

SEQ ID NO: 55 - RNA, 12 nt, Artificial Sequence
  Synthetic construct
  repeat_unit (1)..(12)
uguguguguaug

SEQ ID NO: 56 - RNA, 12 nt, Artificial Sequence
  Synthetic construct
  repeat_unit (1)..(12)
ugugugugugua

SEQ ID NO: 57 - DNA, 70 bp, Unknown
  natural sequence
ggtccagaagcgtgtgtgtgtatgtgtgtgtgtgtgtgtgtgtgtgtgtgtgtgtgtgtgtgtttgtgtg

SEQ ID NO: 58 - RNA, 70 nt, Unknown
  natural sequence
gguccagaagcguguguguguauguguguguguguguguguguguguguguguguguguguguuugugug

SEQ ID NO: 59 - RNA, 34 nt, Unknown
  natural sequence
gagagagcgcgugcagagacuugguggugcauaa

SEQ ID NO: 60 - RNA, 34 nt, Unknown
  natural sequence
uaggagggucagaacugagagugguacaucgcgg

SEQ ID NO: 61 - DNA, 56 bp, Artificial Sequence
  Synthetic construct
cgcgcgcgcgcgcgcgtgtgtgtgtgtgtgtgtgtgtgtgcgcgcgcgcgcgcgcg

SEQ ID NO: 62 - DNA, 20 bp, Artificial Sequence
  Synthetic construct
tgaatgtgtgtgtgtgttgt

SEQ ID NO: 63 - RNA, 20 nt, Artificial Sequence
  Synthetic construct
ugaauguguguguguguugu

SEQ ID NO: 64 - RNA, 36 nt, Artificial Sequence
  Synthetic construct
ugugugugugugugugugugugugugugugugugug

SEQ ID NO: 65 - RNA, 32 nt, Artificial Sequence
  Synthetic construct
ugugugugugugugugugugugugugugugug

SEQ ID NO: 66 - RNA, 28 nt, Artificial Sequence
  Synthetic construct
ugugugugugugugugugugugugugug

SEQ ID NO: 67 - RNA, 22 nt, Artificial Sequence
  Synthetic construct
ugugugugugugugugugugug

SEQ ID NO: 68 - RNA, 20 nt, Artificial Sequence
  Synthetic construct
ugugugugugugugugugug

SEQ ID NO: 69 - RNA, 18 nt, Artificial Sequence
  Synthetic construct
ugugugugugugugugug

SEQ ID NO: 70 - RNA, 16 nt, Artificial Sequence
  Synthetic construct
ugugugugugugugug

SEQ ID NO: 71 - RNA, 14 nt, Artificial Sequence
  Synthetic construct
ugugugugugugug

SEQ ID NO: 72 - RNA, 12 nt, Artificial Sequence
  Synthetic construct
ugugugugugug

SEQ ID NO: 73 - RNA, 10 nt, Artificial Sequence
  Synthetic construct
ugugugugug

SEQ ID NO: 74 - DNA, 24 bp, Artificial Sequence
  Synthetic construct
tgtgtgtgtgtgtgtgtgtgtgtg

SEQ ID NO: 75 - DNA, 36 bp, Artificial Sequence
  Synthetic construct
tgtgtgtgtgtgtgtgtgtgtgtgtgtgtgtgtgtg

SEQ ID NO: 76 - DNA, 32 bp, Artificial Sequence
  Synthetic construct
tgtgtgtgtgtgtgtgtgtgtgtgtgtgtgtg

SEQ ID NO: 77 - DNA, 28 bp, Artificial Sequence
  Synthetic construct
tgtgtgtgtgtgtgtgtgtgtgtgtgtg

SEQ ID NO: 78 - DNA, 22 bp, Artificial Sequence
  Synthetic construct
tgtgtgtgtgtgtgtgtgtgtg

SEQ ID NO: 79 - DNA, 20 bp, Artificial Sequence
  Synthetic construct
tgtgtgtgtgtgtgtgtgtg

SEQ ID NO: 80 - DNA, 18 bp, Artificial Sequence
  Synthetic construct
tgtgtgtgtgtgtgtgtg

SEQ ID NO: 81 - DNA, 16 bp, Artificial Sequence
  Synthetic construct
tgtgtgtgtgtgtgtg

SEQ ID NO: 82 - DNA, 14 bp, Artificial Sequence
  Synthetic construct
tgtgtgtgtgtgtg

SEQ ID NO: 83 - DNA, 12 bp, Artificial Sequence
  Synthetic construct
tgtgtgtgtgtg

SEQ ID NO: 84 - DNA, 10 bp, Artificial Sequence
  Synthetic construct
tgtgtgtgtg

SEQ ID NO: 85 - DNA, 41 bp, Artificial Sequence
  Synthetic construct
gtgtgtgtgtgtgtgtgtgtgtgtgtgtgtgtgtgtgtatg

SEQ ID NO: 86 - DNA, 21 bp, Artificial Sequence
  Synthetic construct
gtggttgtgtgtgtgtggtat

SEQ ID NO: 87 - RNA, 41 nt, Artificial Sequence
  Synthetic construct
guguguguguguguguguguguguguguguguguguguaug

SEQ ID NO: 88 - RNA, 21 nt, Artificial Sequence
  Synthetic construct
gugguugugugugugugguau

SEQ ID NO: 89 - DNA, 28 bp, Artificial Sequence
  Synthetic construct
cgcgcgcgcgcgcgcgcgcgcgcgcgcg

SEQ ID NO: 90 - DNA, 24 bp, Artificial Sequence
  Synthetic construct
cgcgcgcgcgcgcgcgcgcgcgcg

SEQ ID NO: 91 - DNA, 20 bp, Artificial Sequence
  Synthetic construct
cgcgcgcgcgcgcgcgcgcg

SEQ ID NO: 92 - DNA, 16 bp, Artificial Sequence
  Synthetic construct
cgcgcgcgcgcgcgcg

SEQ ID NO: 93 - DNA, 14 bp, Artificial Sequence
  Synthetic construct
cgcgcgcgcgcgcg

SEQ ID NO: 94 - DNA, 12 bp, Artificial Sequence
  Synthetic construct
cgcgcgcgcgcg

SEQ ID NO: 95 - DNA, 10 bp, Artificial Sequence
  Synthetic construct
cgcgcgcgcg

SEQ ID NO: 96 - RNA, 48 nt, Unknown
  natural sequence
gagguggcuauggagguggcuauggagguggcuauggagguggcuaug

SEQ ID NO: 97 - RNA, 24 nt, Unknown
  natural sequence
gacugaaaaagguggguuucuuuu

SEQ ID NO: 98 - RNA, 25 nt, Unknown
  natural sequence
cuaggauggagguggggaaugguac

SEQ ID NO: 99 - RNA, 48 nt, Artificial Sequence
  Synthetic construct
auugaggagcagcagagaaguuggagugaaggcagagagggguuaagg

SEQ ID NO: 100 - RNA, 48 nt, Artificial Sequence
  Synthetic construct
auugaggagcagcagagaaguuggaaaaaaaaaaaaaaaaaaaaaaaa

SEQ ID NO: 101 - RNA, 48 nt, Artificial Sequence
  Synthetic construct
aaaaaaaaaaaaaaaaaaaaaaaaagugaaggcagagagggguuaagg

SEQ ID NO: 102 - RNA, 39 nt, Unknown
  natural sequence
accaugaucacgaaggugguuuucccagggcgaggcuua

SEQ ID NO: 103 - RNA, 43 nt, Unknown
  natural sequence
cuccggaugugcugaccccugcgauuuccccaaaugugggaaa

SEQ ID NO: 104 - RNA, 28 nt, Unknown
  natural sequence
gaaaauuaauguguguguguggaaaauu

SEQ ID NO: 105 - RNA, 25 nt, Unknown
  natural sequence
uuguauuuugagcuaguuuggugau

SEQ ID NO: 106 - RNA, 24 nt, Artificial Sequence
  Synthetic construct
ucagagacaucaucagagacauca

SEQ ID NO: 107 - RNA, 24 nt, Artificial Sequence
  Synthetic construct
ggugagcacagaggugagcacaga

SEQ ID NO: 108 - RNA, 24 nt, Artificial Sequence
  Synthetic construct
ccaaucuuccuuccaaucuuccuu

SEQ ID NO: 109 - RNA, 24 nt, Artificial Sequence
  Synthetic construct
gauggauuccaggauggauuccag

SEQ ID NO: 110 - RNA, 24 nt, Artificial Sequence
  Synthetic construct
aaacggucugauaaacggucugau

SEQ ID NO: 111 - RNA, 40 nt, Artificial Sequence
  Synthetic construct
augucgcagaaugucgcagaaugucgcagaaugucgcaga

SEQ ID NO: 112 - RNA, 40 nt, Artificial Sequence
  Synthetic construct
aaccuucguaaaccuucguaaaccuucguaaaccuucgua

SEQ ID NO: 113 - RNA, 24 nt, Artificial Sequence
  Synthetic construct
cgcuggcauccacgcuggcaucca

SEQ ID NO: 114 - RNA, 24 nt, Artificial Sequence
  Synthetic construct
aaagcggcgaugaaagcggcgaug

SEQ ID NO: 115 - RNA, 24 nt, Artificial Sequence
  Synthetic construct
uauugauccgguuauugauccggu

SEQ ID NO: 116 - RNA, 50 nt, Artificial Sequence
  Synthetic construct
cmumamgmgmamumgmgmamgmgmumgmgmgmgmamamumgmgmumamcm

SEQ ID NO: 117 - RNA, 24 nt, Artificial Sequence
  Synthetic construct
gagguggcuauggagguggcuaug

SEQ ID NO: 118 - RNA, 24 nt, Artificial Sequence
  Synthetic construct
gugguggcuauggagguggcuaug

SEQ ID NO: 119 - RNA, 48 nt, Artificial Sequence
  Synthetic construct
ucagagacaucaucagagacaucaucagagacaucaucagagacauca

SEQ ID NO: 120 - DNA, 112 bp, Artificial Sequence
  Synthetic construct
cmgmcmgmcmgmcmgmcmgmcmgmcmgmcmgmamcmamcmamcmamcmamcmamcmamcmamcmamcmamcmamcmamcmcmgmcmgmcmgmcmgmcmgmcmgmcmgmcmgm

SEQ ID NO: 121 - RNA, 24 nt, Artificial Sequence
  Synthetic construct
uguauuuugagcuaguuugcugau